European Patent Application EP 4 803 550 A1, published September 9, 2026. Title: 一种预防或治疗B 群脑膜炎奈瑟菌相关疾病的免疫组合物产品及其制备方法. Applicant: 烟台派诺生物技术有限公司. The sequence listing filed with the application follows.

SEQUENCE LISTING (75 sequences)

SEQ ID NO: 1 - protein, 545 aa, synthetic construct
SSGSGSGGGGVAADIGTGLADALTAPLDHKDKGLKSLTLEDSISQNGTLTLSAQGAEKTFKVGDKDNSLNTGKLKNDKISRFDFVQKIEVDGQTITLASGEFQIYKQDHSAVVALQIEKINNPDKIDSLINQRSFLVSGLGGEHTSFDKLPKDVMATYRGTAFGSDDAGGKLTYTIDFAAKQGHGKIEHLKSPELNVDLAVAYIKPDEKHHAVISGSVLYNQDEKGSYSLGIFGEKAQEVAGSAEVETANGIHHIGLAAKQGSSGGGGSGGGGVTADIGTGLADALTAPLDHKDKGLKSLTLEDSISQNGTLTLSAQGAEKTYGNGDSLNTGKLKNDKVSRFDFIRQIEVDGQLITLESGEFQVYKQSHSALTALQTEQEQDPEHSEKMVAKRRFRIGDIAGEHTAFNQLPDGKAEYHGKAFSSDDAGGKLTYTIDFAAKQGHGKIEHLKTPEQNVELAAAELKADEKSHAVILGDTRYGSEEKGTYHLALFGDRAQEIAGSATVKIGEKVHEIGIAGKQGSGGSGAHIVMVDAYKPTKHHHHHH

SEQ ID NO: 2 - protein, 539 aa, synthetic construct
SSGSGSGGGGVAADIGTGLADALTAPLDHKDKGLKSLTLEDSISQNGTLTLSAQGAEKTFKVGDKDNSLNTGKLKNDKISRFDFVQKIEVDGQTITLASGEFQIYKQDHSAVVALQIEKINNPDKIDSLINQRSFLVSGLGGEHTSFDKLPKDVMATYRGTAFGSDDAGGKLTYTIDFAAKQGHGKIEHLKSPELNVDLAVAYIKPDEKHHAVISGSVLYNQDEKGSYSLGIFGEKAQEVAGSAEVETANGIHHIGLAAKQGSGGGGVTADIGTGLADALTAPLDHKDKGLKSLTLEDSISQNGTLTLSAQGAEKTYGNGDSLNTGKLKNDKVSRFDFIRQIEVDGQLITLESGEFQVYKQSHSALTALQTEQEQDPEHSEKMVAKRRFRIGDIAGEHTAFNQLPDGKAEYHGKAFSSDDAGGKLTYTIDFAAKQGHGKIEHLKTPEQNVELAAAELKADEKSHAVILGDTRYGSEEKGTYHLALFGDRAQEIAGSATVKIGEKVHEIGIAGKQGSGGSGAHIVMVDAYKPTKHHHHHH

SEQ ID NO: 3 - protein, 526 aa, synthetic construct
HHHHHHSSGSGSGGGGVAADIGTGLADALTAPLDHKDKGLKSLTLEDSISQNGTLTLSAQGAEKTFKVGDKDNSLNTGKLKNDKISRFDFVQKIEVDGQTITLASGEFQIYKQDHSAVVALQIEKINNPDKIDSLINQRSFLVSGLGGEHTSFDKLPKDVMATYRGTAFGSDDAGGKLTYTIDFAAKQGHGKIEHLKSPELNVDLAVAYIKPDEKHHAVISGSVLYNQDEKGSYSLGIFGEKAQEVAGSAEVETANGIHHIGLAAKQGSSGGGGSGGGGVTADIGTGLADALTAPLDHKDKGLKSLTLEDSISQNGTLTLSAQGAEKTYGNGDSLNTGKLKNDKVSRFDFIRQIEVDGQLITLESGEFQVYKQSHSALTALQTEQEQDPEHSEKMVAKRRFRIGDIAGEHTAFNQLPDGKAEYHGKAFSSDDAGGKLTYTIDFAAKQGHGKIEHLKTPEQNVELAAAELKADEKSHAVILGDTRYGSEEKGTYHLALFGDRAQEIAGSATVKIGEKVHEIGIAGKQ

SEQ ID NO: 4 - protein, 551 aa, synthetic construct
HHHHHHSSGSGSGGGGVAADIGTGLADALTAPLDHKDKGLKSLTLEDSISQNGTLTLSAQGAEKTFKVGDKDNSLNTGKLKNDKISRFDFVQKIEVDGQTITLASGEFQIYKQDHSAVVALQIEKINNPDKIDSLINQRSFLVSGLGGEHTSFDKLPKDVMATYRGTAFGSDDAGGKLTYTIDFAAKQGHGKIEHLKSPELNVDLAVAYIKPDEKHHAVISGSVLYNQDEKGSYSLGIFGEKAQEVAGSAEVETANGIHHIGLAAKQGGSGGSGGSGGSAHIVMVDAYKPTKGSSGGGGSGGGGVTADIGTGLADALTAPLDHKDKGLKSLTLEDSISQNGTLTLSAQGAEKTYGNGDSLNTGKLKNDKVSRFDFIRQIEVDGQLITLESGEFQVYKQSHSALTALQTEQEQDPEHSEKMVAKRRFRIGDIAGEHTAFNQLPDGKAEYHGKAFSSDDAGGKLTYTIDFAAKQGHGKIEHLKTPEQNVELAAAELKADEKSHAVILGDTRYGSEEKGTYHLALFGDRAQEIAGSATVKIGEKVHEIGIAGKQ

SEQ ID NO: 5 - protein, 286 aa, synthetic construct
SSGSGSGGGGVAADIGTGLADALTAPLDHKDKGLKSLTLEDSISQNGTLTLSAQGAEKTFKVGDKDNSLNTGKLKNDKISRFDFVQKIEVDGQTITLASGEFQIYKQDHSAVVALQIEKINNPDKIDSLINQRSFLVSGLGGEHTSFDKLPKDVMATYRGTAFGSDDAGGKLTYTIDFAAKQGHGKIEHLKSPELNVDLAVAYIKPDEKHHAVISGSVLYNQDEKGSYSLGIFGEKAQEVAGSAEVETANGIHHIGLAAKQGSGGSGAHIVMVDAYKPTKHHHHHH

SEQ ID NO: 6 - protein, 283 aa, synthetic construct
SSGGGGSGGGGVTADIGTGLADALTAPLDHKDKGLKSLTLEDSISQNGTLTLSAQGAEKTYGNGDSLNTGKLKNDKVSRFDFIRQIEVDGQLITLESGEFQVYKQSHSALTALQTEQEQDPEHSEKMVAKRRFRIGDIAGEHTAFNQLPDGKAEYHGKAFSSDDAGGKLTYTIDFAAKQGHGKIEHLKTPEQNVELAAAELKADEKSHAVILGDTRYGSEEKGTYHLALFGDRAQEIAGSATVKIGEKVHEIGIAGKQGSGGSGAHIVMVDAYKPTKHHHHHH

SEQ ID NO: 7 - protein, 284 aa, synthetic construct
SSGGGGSGGGGVTADIGTGLADALTAPLDHKDKGLKSLTLEDSISQNGTLTLSAQGAEKTYGNGDSLNTGKLKNDKVSRFDFIRQIEVDGQLITLESGEFQVYKQSHSALTALQTEQEQDPEHSEKMVAKRRFRIGDIAGEHTSFDKLPKDVMATYRGTAFGSDDAGGKLTYTIDFAAKQGHGKIEHLKSPELNVDLAVAYIKPDEKHHAVISGSVLYNQDEKGSYSLGIFGEKAQEVAGSAEVETANGIHHIGLAAKQGSGGSGAHIVMVDAYKPTKHHHHHH

SEQ ID NO: 8 - protein, 278 aa, synthetic construct
SSGGGGVAADIGAGLADALTAPLDHKDKSLQSLTLDQSVRKNEKLKLAAQGAEKTYGNGDSLNTGKLKNDKVSRFDFIRQIEVDGQLITLESGEFQIYKQDHSAVVALQIEKINNPDKIDSLINQRSFLVSGLGGEHTAFNQLPDGKAEYHGKAFSSDDAGGKLTYTIDFAAKQGHGKIEHLKTPEQNVELAAAELKADEKSHAVILGDTRYGSEEKGTYHLALFGDRAQEIAGSATVKIGEKVHEIGIAGKQGSGGSGAHIVMVDAYKPTKHHHHHH

SEQ ID NO: 9 - protein, 285 aa, synthetic construct
SSGSGSGGGGVAADIGTGLADALTAPLDHKDKGLKSLTLEDSISQNGTLTLSAQGAEKTFKVGDKDNSLNTGKLKNDKISRFDFVQKIEVDGQTITLASGEFQIYKQDHSAVVALQIEKINNPDKIDSLINQRSFLVSGLGGEHTAFNQLPSGKAEYHGKAFSSDDAGGKLTYTIDFAAKQGHGKIEHLKTPEQNVELASAELKADEKSHAVILGDTRYGSEEKGTYHLALFGDRAQEIAGSATVKIREKVHEIGIAGKQGSGGSGAHIVMVDAYKPTKHHHHHH

SEQ ID NO: 10 - protein, 264 aa, synthetic construct
HHHHHHSSGGGGSGGGGVTADIGTGLADALTAPLDHKDKGLKSLTLEDSISQNGTLTLSAQGAEKTYGNGDSLNTGKLKNDKVSRFDFIRQIEVDGQLITLESGEFQVYKQSHSALTALQTEQEQDPEHSGKMVAKRRFRIGDIAGEHTAFNQLPDGKAEYHGKAFSSDDAGGKLTYTIDFAAKQGHGKIEHLKTPEQNVELAAAELKADEKSHAVILGDTRYGSEEKGTYHLALFGDRAQEIAGSATVKIGEKVHEIGIAGKQ

SEQ ID NO: 11 - protein, 264 aa, synthetic construct
HHHHHHSSGGGGSGGGGVTADIGTGLADALTAPLDHKDKGLKSLTLEDSISQNGTLTLSAQGAEKTYGNGDSLNTGKLKNDKVSRFDFIRQIEVDGQLITLESGEFQVYKQSHSALTALQTEQEQDPEHSGKMVAKRRFRIGDIAGEHTAFNQLPDGKAEYHGKAFSSDDAGGKLTYTIDFAKKQGHGRIEHLKTPEQNVELAAAELKADEKSHAVILGDTRYGSEEKGTYHLALFGDRAQEIAGSATVKIGEKVHEIGIAGKQ

SEQ ID NO: 12 - protein, 546 aa, synthetic construct
SSGGGGSGGGGVTADIGTGLADALTAPLDHKDKGLKSLTLEDSISQNGTLTLSAQGAEKTYGNGDSLNTGKLKNDKVSRFDFIRQIEVDGQLITLESGEFQVYKQSHSALTALQTEQEQDPEHSEKMVAKRRFRIGDIAGEHTAFNQLPDGKAEYHGKAFSSDDAGGKLTYTIDFAAKQGHGKIEHLKTPEQNVELAAAELKADEKSHAVILGDTRYGSEEKGTYHLALFGDRAQEIAGSATVKIGEKVHEIGIAGKQGGSSGSGSGGGGVAADIGTGLADALTAPLDHKDKGLKSLTLEDSISQNGTLTLSAQGAEKTFKVGDKDNSLNTGKLKNDKISRFDFVQKIEVDGQTITLASGEFQIYKQDHSAVVALQIEKINNPDKIDSLINQRSFLVSGLGGEHTSFDKLPKDVMATYRGTAFGSDDAGGKLTYTIDFAAKQGHGKIEHLKSPELNVDLAVAYIKPDEKHHAVISGSVLYNQDEKGSYSLGIFGEKAQEVAGSAEVETANGIHHIGLAAKQGSGGSGAHIVMVDAYKPTKHHHHHH

SEQ ID NO: 13 - protein, 540 aa, synthetic construct
SSGGGGSGGGGVTADIGTGLADALTAPLDHKDKGLKSLTLEDSISQNGTLTLSAQGAEKTYGNGDSLNTGKLKNDKVSRFDFIRQIEVDGQLITLESGEFQVYKQSHSALTALQTEQEQDPEHSEKMVAKRRFRIGDIAGEHTAFNQLPDGKAEYHGKAFSSDDAGGKLTYTIDFAAKQGHGKIEHLKTPEQNVELAAAELKADEKSHAVILGDTRYGSEEKGTYHLALFGDRAQEIAGSATVKIGEKVHEIGIAGKQGSGGGGVAADIGTGLADALTAPLDHKDKGLKSLTLEDSISQNGTLTLSAQGAEKTFKVGDKDNSLNTGKLKNDKISRFDFVQKIEVDGQTITLASGEFQIYKQDHSAVVALQIEKINNPDKIDSLINQRSFLVSGLGGEHTSFDKLPKDVMATYRGTAFGSDDAGGKLTYTIDFAAKQGHGKIEHLKSPELNVDLAVAYIKPDEKHHAVISGSVLYNQDEKGSYSLGIFGEKAQEVAGSAEVETANGIHHIGLAAKQGSGGSGAHIVMVDAYKPTKHHHHHH

SEQ ID NO: 14 - protein, 535 aa, synthetic construct
VAADIGTGLADALTAPLDHKDKGLKSLTLEDSISQNGTLTLSAQGAEKTFKVGDKDNSLNTGKLKNDKISRFDFVQKIEVDGQTITLASGEFQIYKQDHSAVVALQIEKINNPDKIDSLINQRSFLVSGLGGEHTSFDKLPKDVMATYRGTAFGSDDAGGKLTYTIDFAAKQGHGKIEHLKSPELNVDLAVAYIKPDEKHHAVISGSVLYNQDEKGSYSLGIFGEKAQEVAGSAEVETANGIHHIGLAAKQGSSGGGGSGGGGVTADIGTGLADALTAPLDHKDKGLKSLTLEDSISQNGTLTLSAQGAEKTYGNGDSLNTGKLKNDKVSRFDFIRQIEVDGQLITLESGEFQVYKQSHSALTALQTEQEQDPEHSEKMVAKRRFRIGDIAGEHTAFNQLPDGKAEYHGKAFSSDDAGGKLTYTIDFAAKQGHGKIEHLKTPEQNVELAAAELKADEKSHAVILGDTRYGSEEKGTYHLALFGDRAQEIAGSATVKIGEKVHEIGIAGKQGSGGSGAHIVMVDAYKPTKHHHHHH

SEQ ID NO: 15 - protein, 477 aa, synthetic construct
LNTGKLKNDKISRFDFVQKIEVDGQTITLASGEFQIYKQDHSAVVALQIEKINNPDKIDSLINQRSFLVSGLGGEHTSFDKLPKDVMATYRGTAFGSDDAGGKLTYTIDFAAKQGHGKIEHLKSPELNVDLAVAYIKPDEKHHAVISGSVLYNQDEKGSYSLGIFGEKAQEVAGSAEVETANGIHHIGLAAKQGSSGGGGSGGGGVTADIGTGLADALTAPLDHKDKGLKSLTLEDSISQNGTLTLSAQGAEKTYGNGDSLNTGKLKNDKVSRFDFIRQIEVDGQLITLESGEFQVYKQSHSALTALQTEQEQDPEHSEKMVAKRRFRIGDIAGEHTAFNQLPDGKAEYHGKAFSSDDAGGKLTYTIDFAAKQGHGKIEHLKTPEQNVELAAAELKADEKSHAVILGDTRYGSEEKGTYHLALFGDRAQEIAGSATVKIGEKVHEIGIAGKQGSGGSGAHIVMVDAYKPTKHHHHHH

SEQ ID NO: 16 - protein, 543 aa, synthetic construct
SSGSGSGGGGVAADIGTGLADALTAPLDHKDKGLKSLTLEDSISQNGTLTLSAQGAEKTFKVGDKDNSLNTGKLKNDKISRFDFVQKIEVDGQTITLASGEFQIYKQDHSAVVALQIEKINNPDKIDSLINQRSFLVSGLGGEHTSFDKLPKDVMATYRGTAFGSDDAGGKLTYTIDFAAKQGHGKIEHLKSPELNVDLAVAYIKPDEKHHAVISGSVLYNQDEKGSYSLGIFGEKAQEVAGSAEVETANGIHHIGLAAKQGGSGGEAAAKVTADIGTGLADALTAPLDHKDKGLKSLTLEDSISQNGTLTLSAQGAEKTYGNGDSLNTGKLKNDKVSRFDFIRQIEVDGQLITLESGEFQVYKQSHSALTALQTEQEQDPEHSEKMVAKRRFRIGDIAGEHTAFNQLPDGKAEYHGKAFSSDDAGGKLTYTIDFAAKQGHGKIEHLKTPEQNVELAAAELKADEKSHAVILGDTRYGSEEKGTYHLALFGDRAQEIAGSATVKIGEKVHEIGIAGKQGSGGSGAHIVMVDAYKPTKHHHHHH

SEQ ID NO: 17 - protein, 543 aa, synthetic construct
SSGSGSGGGGVAADIGTGLADALTAPLDHKDKGLKSLTLEDSISQNGTLTLSAQGAEKTFKVGDKDNSLNTGKLKNDKISRFDFVQKIEVDGQTITLASGEFQIYKQDHSAVVALQIEKINNPDKIDSLINQRSFLVSGLGGEHTSFDKLPKDVMATYRGTAFGSDDAGGKLTYTIDFAAKQGHGKIEHLKSPELNVDLAVAYIKPDEKHHAVISGSVLYNQDEKGSYSLGIFGEKAQEVAGSAEVETANGIHHIGLAAKQEAAAKEAAAKVTADIGTGLADALTAPLDHKDKGLKSLTLEDSISQNGTLTLSAQGAEKTYGNGDSLNTGKLKNDKVSRFDFIRQIEVDGQLITLESGEFQVYKQSHSALTALQTEQEQDPEHSEKMVAKRRFRIGDIAGEHTAFNQLPDGKAEYHGKAFSSDDAGGKLTYTIDFAAKQGHGKIEHLKTPEQNVELAAAELKADEKSHAVILGDTRYGSEEKGTYHLALFGDRAQEIAGSATVKIGEKVHEIGIAGKQGSGGSGAHIVMVDAYKPTKHHHHHH

SEQ ID NO: 18 - protein, 532 aa, synthetic construct
SSGGGGVAADIGAGLADALTAPLDHKDKSLQSLTLDQSVRKNEKLKLAAQGAEKTYGNGDSLNTGKLKNDKVSRFDFIRQIEVDGQLITLESGEFQIYKQDHSAVVALQIEKINNPDKIDSLINQRSFLVSGLGGEHTSFDKLPKDVMATYRGTAFGSDDAGGKLTYTIDFAAKQGHGKIEHLKSPELNVDLAVAYIKPDEKHHAVISGSVLYNQDEKGSYSLGIFGEKAQEVAGSAEVETANGIHHIGLAAKQGSGGGGVTADIGTGLADALTAPLDHKDKGLKSLTLEDSISQNGTLTLSAQGAEKTYGNGDSLNTGKLKNDKVSRFDFIRQIEVDGQLITLESGEFQVYKQSHSALTALQTEQEQDPEHSEKMVAKRRFRIGDIAGEHTAFNQLPSGKAEYHGKAFSSDDAGGKLTYTIDFAAKQGHGKIEHLKTPEQNVELASAELKADEKSHAVILGDTRYGSEEKGTYHLALFGDRAQEIAGSATVKIREKVHEIGIAGKQGSGGSGAHIVMVDAYKPTKHHHHHH

SEQ ID NO: 19 - protein, 548 aa, synthetic construct
SSGSGSGGGGVAADIGTGLADALTAPLDHKDKGLKSLTLEDSISQNGTLTLSAQGAEKTFKVGDKDNSLNTGKLKNDKISRFDFVQKIEVDGQTITLASGEFQIYKQDHSAVVALQIEKINNPDKIDSLINQRSFLVSGLGGEHTSFDKLPKDVMATYRGTAFGSDDAGGKLTYTIDFAAKQGHGKIEHLKSPELNVDLAVAYIKPDEKHHAVISGSVLYNQDEKGSYSLGIFGEKAQEVAGSAEVETANGIHHIGLAAKQEAAAKEAAAKEAAAKVTADIGTGLADALTAPLDHKDKGLKSLTLEDSISQNGTLTLSAQGAEKTYGNGDSLNTGKLKNDKVSRFDFIRQIEVDGQLITLESGEFQVYKQSHSALTALQTEQEQDPEHSEKMVAKRRFRIGDIAGEHTAFNQLPDGKAEYHGKAFSSDDAGGKLTYTIDFAAKQGHGKIEHLKTPEQNVELAAAELKADEKSHAVILGDTRYGSEEKGTYHLALFGDRAQEIAGSATVKIGEKVHEIGIAGKQGSGGSGAHIVMVDAYKPTKHHHHHH

SEQ ID NO: 20 - protein, 553 aa, synthetic construct
SSGSGSGGGGVAADIGTGLADALTAPLDHKDKGLKSLTLEDSISQNGTLTLSAQGAEKTFKVGDKDNSLNTGKLKNDKISRFDFVQKIEVDGQTITLASGEFQIYKQDHSAVVALQIEKINNPDKIDSLINQRSFLVSGLGGEHTSFDKLPKDVMATYRGTAFGSDDAGGKLTYTIDFAAKQGHGKIEHLKSPELNVDLAVAYIKPDEKHHAVISGSVLYNQDEKGSYSLGIFGEKAQEVAGSAEVETANGIHHIGLAAKQEAAAKEAAAKEAAAKEAAAKVTADIGTGLADALTAPLDHKDKGLKSLTLEDSISQNGTLTLSAQGAEKTYGNGDSLNTGKLKNDKVSRFDFIRQIEVDGQLITLESGEFQVYKQSHSALTALQTEQEQDPEHSEKMVAKRRFRIGDIAGEHTAFNQLPDGKAEYHGKAFSSDDAGGKLTYTIDFAAKQGHGKIEHLKTPEQNVELAAAELKADEKSHAVILGDTRYGSEEKGTYHLALFGDRAQEIAGSATVKIGEKVHEIGIAGKQGSGGSGAHIVMVDAYKPTKHHHHHH

SEQ ID NO: 21 - protein, 536 aa, synthetic construct
SSGGGGVAADIGAGLADALTAPLDHKDKSLQSLTLDQSVRKNEKLKLAAQGAEKTYGNGDSLNTGKLKNDKVSRFDFIRQIEVDGQLITLESGEFQIYKQDHSAVVALQIEKINNPDKIDSLINQRSFLVSGLGGEHTSFDKLPKDVMATYRGTAFGSDDAGGKLTYTIDFAAKQGHGKIEHLKSPELNVDLAVAYIKPDEKHHAVISGSVLYNQDEKGSYSLGIFGEKAQEVAGSAEVETANGIHHIGLAAKQEAAAKEAAAKVTADIGTGLADALTAPLDHKDKGLKSLTLEDSISQNGTLTLSAQGAEKTYGNGDSLNTGKLKNDKVSRFDFIRQIEVDGQLITLESGEFQVYKQSHSALTALQTEQEQDPEHSEKMVAKRRFRIGDIAGEHTAFNQLPSGKAEYHGKAFSSDDAGGKLTYTIDFAAKQGHGKIEHLKTPEQNVELASAELKADEKSHAVILGDTRYGSEEKGTYHLALFGDRAQEIAGSATVKIREKVHEIGIAGKQGSGGSGAHIVMVDAYKPTKHHHHHH

SEQ ID NO: 22 - protein, 541 aa, synthetic construct
SSGGGGVAADIGAGLADALTAPLDHKDKSLQSLTLDQSVRKNEKLKLAAQGAEKTYGNGDSLNTGKLKNDKVSRFDFIRQIEVDGQLITLESGEFQIYKQDHSAVVALQIEKINNPDKIDSLINQRSFLVSGLGGEHTSFDKLPKDVMATYRGTAFGSDDAGGKLTYTIDFAAKQGHGKIEHLKSPELNVDLAVAYIKPDEKHHAVISGSVLYNQDEKGSYSLGIFGEKAQEVAGSAEVETANGIHHIGLAAKQEAAAKEAAAKEAAAKVTADIGTGLADALTAPLDHKDKGLKSLTLEDSISQNGTLTLSAQGAEKTYGNGDSLNTGKLKNDKVSRFDFIRQIEVDGQLITLESGEFQVYKQSHSALTALQTEQEQDPEHSEKMVAKRRFRIGDIAGEHTAFNQLPSGKAEYHGKAFSSDDAGGKLTYTIDFAAKQGHGKIEHLKTPEQNVELASAELKADEKSHAVILGDTRYGSEEKGTYHLALFGDRAQEIAGSATVKIREKVHEIGIAGKQGSGGSGAHIVMVDAYKPTKHHHHHH

SEQ ID NO: 23 - protein, 546 aa, synthetic construct
SSGGGGVAADIGAGLADALTAPLDHKDKSLQSLTLDQSVRKNEKLKLAAQGAEKTYGNGDSLNTGKLKNDKVSRFDFIRQIEVDGQLITLESGEFQIYKQDHSAVVALQIEKINNPDKIDSLINQRSFLVSGLGGEHTSFDKLPKDVMATYRGTAFGSDDAGGKLTYTIDFAAKQGHGKIEHLKSPELNVDLAVAYIKPDEKHHAVISGSVLYNQDEKGSYSLGIFGEKAQEVAGSAEVETANGIHHIGLAAKQEAAAKEAAAKEAAAKEAAAKVTADIGTGLADALTAPLDHKDKGLKSLTLEDSISQNGTLTLSAQGAEKTYGNGDSLNTGKLKNDKVSRFDFIRQIEVDGQLITLESGEFQVYKQSHSALTALQTEQEQDPEHSEKMVAKRRFRIGDIAGEHTAFNQLPSGKAEYHGKAFSSDDAGGKLTYTIDFAAKQGHGKIEHLKTPEQNVELASAELKADEKSHAVILGDTRYGSEEKGTYHLALFGDRAQEIAGSATVKIREKVHEIGIAGKQGSGGSGAHIVMVDAYKPTKHHHHHH

SEQ ID NO: 24 - DNA, 1641 bp, synthetic construct
  source 1..1641: mol_type = other DNA
tctagcggttcaggaagtggcggagggggggtggcagctgacatcggcactggtctggcggacgctctgaccgctccgctggaccacaaggacaaaggtttgaaaagcctgactttggaagattcgatctctcagaatggtacgctgaccctcagcgcgcaaggcgcggagaagacctttaaagttggtgataaggacaacagcttgaacaccggtaaactgaaaaacgataagattagccgcttcgacttcgtgcagaaaatcgaagtggacggtcagaccattacccttgcgagcggcgagttccagatttacaagcaggatcatagtgcggttgtcgcattacaaatcgaaaaaatcaataatccggataagattgattctctcatcaaccaacgtagcttcttggttagcggcctgggtggcgaacacaccagctttgataagctgccaaaagatgtcatggcaacctaccgtggtacggcgttcggctcggacgacgcgggtggcaaattaacttacaccattgactttgcagcgaagcagggccatggcaaaatcgagcacctgaagtccccggaactgaacgtggacctggcagtggcgtacatcaaaccggacgaaaagcatcatgctgtgatcagcggttcggtgctgtataaccaagatgagaaaggcagctatagcctgggtatttttggcgagaaggcgcaggaggtggcgggttccgccgaggttgaaaccgcgaatggcatccatcacattgggttggcggcaaaacagggctctagcggaggtggtggttccggtggtggcggtgttaccgcggacatcggtaccggtttggcggatgcgcttacggcaccgctggatcacaaagacaagggtctgaagtccttgaccttggaggactccatttcgcaaaacggcaccctgacgcttagcgctcaaggcgcagaaaagacctacggcaatggtgactcactgaacaccggtaaactgaagaacgacaaagttagccgcttcgactttatccgtcagattgaggttgatggtcagctgattaccctggaaagcggggagtttcaggtatataagcaatcccattccgcgctgactgccctgcagaccgaacaagaacaggacccggagcactccgaaaaaatggttgcaaagcgccgttttcgtattggtgacattgcgggcgagcacaccgcgttcaaccagctgcctgatggtaaagccgagtatcacggcaaggccttcagcagcgatgacgccgggggtaagttaacgtacaccattgactttgccgcgaagcaaggtcacgggaaaatcgagcacctgaagacaccggagcaaaatgtcgagttggctgcggcagagctgaaggctgacgaaaagagccatgcagtcatcctgggcgatacccgttatggttctgaagaaaagggtacgtaccacctggccttgttcggtgatcgtgcccaagagatcgcgggctctgctaccgttaaaatcggcgaaaaagtgcatgaaatcggtatcgcgggtaaacagggttctggcggctctggcgcccatattgttatggtggacgcatataaaccgaccaaacatcatcaccaccaccactaatga

SEQ ID NO: 25 - DNA, 1623 bp, synthetic construct
  source 1..1623: mol_type = other DNA
tctagcggttcaggaagtggaggcgggggggtggcggcggacatcggtaccggtttagcggacgctctcaccgcaccgctggatcataaggacaaaggcctaaagtccctgaccctggaagacagcattagccagaatggcaccctgaccctgagcgcccagggcgcagagaagacctttaaagttggcgacaaggacaactccttgaacacgggcaagctgaagaacgacaagatctcccgcttcgatttcgtgcagaaaatcgaagttgatggccagaccatcaccttggcgagcggtgagttccagatttataaacaggaccacagcgcggtcgtggctctgcagatcgaaaaaattaacaacccggacaaaatcgactcgctgatcaaccagcgtagctttctggtttccggtctgggcggtgagcacaccagttttgataaactgcctaaagatgttatggcaacctaccgcggtacggcgtttggttcggatgatgcgggcgggaaattgacctatacgatcgatttcgccgcgaagcagggtcatggtaagatcgaacacctaaagtccccggaacttaacgtggacctggcggtggcgtatatcaagccggatgaaaagcatcacgcagtcatcagcggctccgtgctgtacaatcaagacgaaaagggttcttatagcttaggtatcttcggcgagaaagcccaagaggtcgcaggttccgcggaggtcgagacggccaatggtattcatcacattggtcttgcggcaaaacaaggcagcggaggtggcggtgttaccgcggacattggtactggtttggcggacgctctgactgcgccactggaccacaaagataagggcttgaagtcattgaccttggaggatagcattagccaaaatggcaccctgacactgtctgcgcagggtgccgagaagacctacggtaatggggactctctgaacactggcaaacttaaaaacgataaggtgagccgcttcgattttatccgtcaaattgaagtggacggtcagctgattacgctggagagcggcgagtttcaggtttataaacaaagccattccgctctgacggctttgcaaaccgaacaagaacaggacccggagcactctgaaaagatggtggctaaacgtcgtttccgtattggcgacattgcaggtgagcacaccgcgtttaaccagctgccggatggcaaggccgagtatcacggtaaggccttcagcagcgatgacgctggcggtaaattgacgtacaccattgatttcgccgcgaaacaagggcatggtaagatcgagcatttgaagactccggaacaaaatgttgaactggcggccgcggagctgaaggcggacgaaaaatctcatgcagttattctgggcgacacccgttacggtagcgaagagaaaggtacctaccacctggctctgtttggtgacagagcacaggagatcgctggtagcgcgaccgtaaaaattggtgaaaaagttcatgaaatcggtatcgcaggcaagcaaggctcaggcggctctggcgcgcatattgttatggtggatgcgtacaagccgacaaaacaccaccatcaccaccactaatga

SEQ ID NO: 26 - DNA, 1584 bp, synthetic construct
  source 1..1584: mol_type = other DNA
caccatcaccaccaccattcatctggaagtggttcaggtggcggtggcgtggcggctgacatcggcaccggtcttgctgacgctttgacggctccgctggatcataaagacaaaggtctgaaaagcctaaccttggaagatagcatctctcagaatggcactctgacgctgagcgctcagggcgcagagaaaacctttaaagtgggtgacaaggacaacagcctgaacaccggtaagctgaagaatgataaaatcagtagattcgattttgttcagaaaattgaagttgatggccagacgattaccttggccagcggtgagttccagatctacaagcaagatcacagcgcggtagttgccctgcaaattgaaaagatcaacaacccggataaaatcgattctctgataaaccagcgtagctttctggtttctggcttaggcggtgaacacaccagctttgataagttgccgaaagatgtgatggcaacctaccgtggtacggccttcggctcggacgatgctgggggcaagctgacgtacaccattgacttcgcagcgaaacagggtcacggtaaaatcgagcaccttaagtcgccggaattgaatgtggacctggcggttgcgtatattaaaccggatgaaaaacatcacgcagtgatctccggtagcgttctgtataatcaggatgagaagggtagctatagcctgggcatttttggtgaaaaggcgcaggaggtcgcgggttctgcggaggtggagacagcgaatggtattcatcatattggcctggcggcgaagcaaggttccagcggcggtggaggcagcggtggcggcggcgtgacggctgacatcggcaccggtctggcggacgcgctcactgcgccactggaccacaaagacaaaggcctcaagagcttgaccttggaggactcgattagccaaaacggcactttgactttgagcgctcagggtgcagagaagacctacggtaatggcgactccctcaacaccggtaaactgaagaacgataaagttagtcgcttcgatttcatccgccagatcgaggtggacggccaactgattacccttgagagcggtgagttccaagtttataagcaatcccactcggctctgaccgcgctgcagaccgaacaagaacaggacccggagcacagcgaaaagatggttgcgaagcgccgttttcgtatcggagacatcgctggcgagcacaccgcgttcaaccaactgccggacggtaaagcggagtatcatggtaaggcattcagctccgacgacgcaggtggcaaactgacttacaccattgactttgcggcaaaacaaggccacggcaaaatcgagcacctgaaaaccccggaacaaaacgtggaactggcagcggcggaactgaaggccgacgaaaagtcccatgccgtcatcctgggtgacacccgttacggctctgaagaaaaaggtacctaccatctggcactgtttggtgatcgtgcccaggagatcgccggctctgcgaccgtcaaaatcggtgagaaggttcatgaaattggtattgcggggaagcaataatga

SEQ ID NO: 27 - DNA, 1659 bp, synthetic construct
  source 1..1659: mol_type = other DNA
caccatcaccaccaccattcatctggaagtggttccggtggtggtggtgttgccgcggacattggcactggactggccgacgcgctgaccgcgccactggaccacaaggacaagggtctgaaaagcctgacattggaggatagcattagccagaacggtacgttgactttatctgcccaaggcgcggaaaaaacctttaaagtcggtgacaaggacaacagcctcaataccggcaagctgaaaaacgataaaatcagtagattcgactttgtccagaaaatcgaagtggacggtcagacgatcaccttggctagcggtgaatttcagatttataaacaggaccactccgctgtcgtggcactgcagattgaaaagatcaacaacccggacaagatcgatagcctaatcaatcaacgtagctttctggttagcggcctgggcggtgagcacacgagcttcgataaactcccgaaagatgttatggcaacctaccgcggtaccgcgttcggctctgatgatgctggtggcaagctgacgtacaccatcgacttcgcggctaagcaaggccatggcaaaatcgagcacctgaagtccccggaactgaacgttgacctggccgtggcatacattaaaccggatgagaaacatcacgccgtcatctctggctctgttctgtataaccaggatgaaaaaggttcatatagcctgggtatttttggtgaaaaggcacaagaggtggcgggttccgcggaggtggaaaccgcaaatggcatccatcacattggtttggctgcgaagcaaggtggaagtggcggctcggggggttctggcggctccgcgcatattgttatggttgatgcgtataaaccgaccaaaggttcgagcggtgggggtggctctggcggtgggggcgtgaccgcggacatcggcaccggcctggcggacgccttgaccgctccgctggatcacaaagataagggcctgaagtccttaactctcgaagattccatctcccagaatggtaccctgacgcttagcgcgcaaggcgcggagaaaacctacggaaacggtgacagcctgaatactggcaagctgaagaacgataaagtgagccgttttgatttcattcgtcaaatcgaggtggacggccagctgattaccctggaaagcggcgagttccaggtgtacaagcaaagccatagcgcattgaccgcgctgcaaaccgaacaagaacaggacccggaacactcggagaagatggtggcgaagcgccgttttcgtattggtgacatcgccggcgagcacaccgccttcaaccagctgccggatggtaaagctgagtatcacggtaaagcgttcagcagcgacgacgccggtggtaagttgacgtacaccatcgacttcgctgcgaaacaaggtcacggcaaaatcgagcacctgaagaccccggagcagaatgttgaactggcggcagcggagctgaaagctgacgagaagtcgcatgcggtgattctgggtgatacccgttatggttccgaagaaaagggcacctaccatctggcgttgttcggtgaccgcgcacaggagatcgcaggctctgcgaccgttaaaattggtgagaaagttcatgaaattggtattgcaggcaagcagtaatga

SEQ ID NO: 28 - DNA, 864 bp, synthetic construct
  source 1..864: mol_type = other DNA
tctagcggaagtggttcagggggaggcggggtggctgcggacatcggcacgggtctggctgatgcactgactgcgccactggatcataaagacaagggtctgaaaagcctgaccttggaagattccatttcgcaaaacggtactttgaccctgagcgctcagggcgcagaaaaaacctttaaagttggtgataaggacaatagcttgaacaccggtaaactgaagaatgataaaatctctcgttttgacttcgtgcagaaaatcgaggtcgatggtcagaccattaccttggcgagcggcgaatttcagatttataaacaagaccatagcgcggttgttgcgctgcagattgagaagatcaacaacccggacaagatcgacagcctgattaatcaacgttcgttcctggttagcgggctgggtggcgagcataccagcttcgacaagctgccgaaagatgttatggcaacctaccgcggtacggcgtttggcagcgatgatgcgggtggcaagctgacgtacaccatcgacttcgccgcgaaacaaggtcatggtaaaatcgagcacctgaagtccccggaactgaatgttgacctggcggtggcctacattaaaccggacgagaagcaccacgcggtgatctcaggttccgtgctgtataaccaggatgagaaaggcagctatagcttaggtatcttcggcgaaaaggcccaagaagtcgccggttctgcagaggtggaaaccgcgaacggcattcatcacatcggcctcgcggcaaagcagggttccggcggttctggcgctcatattgttatggtggacgcttacaagccgaccaaacatcaccaccaccaccactaatga

SEQ ID NO: 29 - DNA, 855 bp, synthetic construct
  source 1..855: mol_type = other DNA
tcatctggtggagggggaagtggcggagggggtgttaccgccgacatcgggacgggtctggctgacgccttgactgcgccactggatcataaagataaaggtcttaagtcgctgacgttggaggacagtattagccagaacggtaccctgaccctgtctgctcagggcgcagagaaaacctacggcaatggagacagcctgaacaccggtaaactgaagaacgataaggtgagccgttttgatttcatccgtcagattgaagttgacggccagctgattaccttggagagcggcgaatttcaggtgtataagcaaagccactccgcgttgactgcgttacaaaccgaacaagaacaggacccggaacactcggaaaaaatggtcgccaagcgcagattccgcattggcgacatcgcgggcgagcacaccgcgttcaaccagctgccggatggcaaggcggagtatcacggcaaggccttcagctccgatgatgccggcggtaaattgacgtacaccattgattttgcggcgaaacaaggtcatggcaagatcgagcacctcaagaccccggaacagaatgttgagctggcagctgctgagctgaaggcggacgaaaagagccacgctgtgatcctgggggacacccgttatggttccgaggaaaaaggcacgtaccatctggcgttatttggtgaccgtgcacaagagatcgcgggtagcgcaaccgttaaaattggtgagaaagtacatgaaatcggtatcgcgggtaagcaaggctccggcggttctggtgcacatattgtcatggtggacgcgtacaaaccgaccaaacaccatcaccaccaccattaatga

SEQ ID NO: 30 - DNA, 858 bp, synthetic construct
  source 1..858: mol_type = other DNA
tcatctggtggagggggaagtggcggagggggcgtgaccgcggacatcggtacaggcttagcggacgctctgacggctccgctggatcataaggacaaaggcttgaagtcgttgacccttgaggacagcatcagccagaacggcactctgaccctctcggctcaaggtgcggaaaagacctacggcaacggcgacagcctgaataccggtaagctgaagaacgataaagtttctcgtttcgacttcattcgtcaaatcgaagttgatggtcagctgatcaccttggagagcggagagttccaggtgtataaacaaagccatagtgcactgacggcgctgcagaccgaacaagaacaggacccggagcacagcgaaaagatggttgctaaacgtcgctttcgtattggcgacatcgccggtgagcacaccagctttgataaactaccgaaagacgtcatggcaacctaccgcggtactgcctttggttccgatgatgcgggtggtaagctgacgtacaccattgattttgcggcgaagcaaggtcatggtaaaattgagcacctgaagtccccggagctgaacgtggacctggcggtcgcatacatcaaaccggacgaaaaacaccacgccgttattagcggctctgttctgtataaccaggatgagaagggtagctattccctgggtatcttcggtgaaaaggcgcaggaggtggccggttctgcggaagtagaaaccgcgaatggcattcaccacatcggtttggctgcaaagcaaggcagcggtggctccggcgcacatatcgtgatggttgacgcgtacaaaccaacgaaacatcatcaccaccatcactaatga

SEQ ID NO: 31 - DNA, 840 bp, synthetic construct
  source 1..840: mol_type = other DNA
tcaagtggtggaggaggggtagcagctgacatcggtgctggcctggcggacgcgctgacggctccgctggaccataaagataaatccttacagagcttaactctggaccaatcagttcgcaaaaacgaaaaattgaagttggccgcgcagggtgcggaaaaaacgtacggaaacggcgacagcttgaataccggtaagctcaagaacgataaggtctctcgttttgattttatccgtcagattgaggtggacggtcagctgattaccctggaaagcggcgagttccagatttacaagcaagatcatagcgctgtggtggcattgcaaatcgagaagatcaataacccggacaaaatcgacagccttatcaaccagcgtagcttcctggtgtccggtctgggcggtgagcacaccgcgtttaaccagttgccagacggcaaggctgagtatcacggcaaagcgttcagcagcgatgatgcgggcggtaagctgacctacaccatcgacttcgcggcgaaacaaggtcatggcaaaattgagcacctgaagaccccggaacagaatgttgaactggctgcggcggagctgaaggcggatgaaaagtcccatgcggtcattctgggtgatacccgttatggctcggaagagaaaggtacataccatctggccttgtttggtgatcgcgcacaagagatcgccggtagcgccaccgttaaaatcggcgagaaggtgcatgaaattggtattgcaggtaagcaaggctctggcgggtctggtgcccatattgttatggttgacgcatataaaccgacgaaacaccaccaccaccaccactaatga

SEQ ID NO: 32 - DNA, 861 bp, synthetic construct
  source 1..861: mol_type = other DNA
tctagcggaagtggttcaggaggcgggggggtggctgctgatattggtaccggcctggccgacgctctcacggcgccactggatcacaaagataagggcttgaaatcgttgaccctggaagattcaattagccagaacggtactttgaccctatctgcgcaaggtgcggaaaagacgtttaaagttggtgacaaggacaacagccttaatactggtaagctgaagaacgacaaaatcagtcgttttgatttcgtgcagaaaatcgaggtagatggtcaaaccattaccttggcgagcggtgagttccagatctacaaacaagaccacagcgctgtggttgcattacagattgagaagatcaacaacccggataagatcgactccctgattaatcaacgcagcttcctggttagcggcctgggcggcgagcacaccgcgttcaaccagctgccgagcggcaaggccgagtatcatggcaaggcgttttccagcgatgatgcaggtggcaagctgacgtacaccattgactttgccgcgaaacagggtcatggtaagatcgagcacctgaaaaccccggaacagaatgtcgagttggcgtccgcggaactgaaagcagacgagaaaagccacgcagtcatcctgggggacacccgttatggatctgaagagaaaggtacataccatctggcactgttcggcgaccgcgcgcaagagattgccggttcggctaccgttaaaatccgtgaaaaggtgcatgaaatcggaatcgcgggtaagcagggcagcggtggctctggtgcccatattgttatggtggacgcgtataaaccgaccaaacatcaccaccaccatcactaatga

SEQ ID NO: 33 - DNA, 798 bp, synthetic construct
  source 1..798: mol_type = other DNA
caccatcaccaccaccattcaagtggagggggcggttctggtggtggcggagttaccgcggacatcggcacgggcctggcggacgccttgacggctccgctggatcataaagacaaaggtctgaaatccttgaccttggaggactccattagccagaatggtaccctgaccttaagcgctcagggtgcagagaagacctacggcaacggcgactccttgaatacgggcaagttgaagaacgataaagtcagcagatttgacttcatccgccagattgaagttgatggtcagcttatcaccctggaaagcggtgagtttcaggtttataaacagtctcacagcgcgctcactgcgctgcagaccgaacaagagcaagatccagaacactctggcaagatggtggcaaaacgccgttttcgtattggcgacatcgcgggcgagcacaccgcgttcaaccagctgccggatggcaaagcggagtatcatggtaaggcgttcagcagcgatgatgcaggtggtaagctgacgtacaccattgatttcgccgcgaaacaaggtcacggcaagatcgagcacctgaaaaccccggagcaaaacgtggaactggcggcagctgagctgaaggcggacgaaaagagccacgctgtgattctgggtgacacccgttatggttcggaagaaaagggtacttaccatctggcgctgtttggtgaccgtgcacaagagatcgccggctcggctaccgttaaaatcggcgagaaagtgcatgaaatcggcattgccggcaagcaataatga

SEQ ID NO: 34 - DNA, 798 bp, synthetic construct
  source 1..798: mol_type = other DNA
caccaccatcaccaccattcaagtggagggggcggttcgggcggtggcggggtgaccgcggacatcggtacgggtctggctgacgccctcacggctccgctggatcataaagataaaggtttgaagtccctgaccctggaagatagtatttcgcaaaatggtacgttaaccctgagcgcgcagggtgcagagaagacctacggaaacggcgacagcctgaacaccggtaagctgaagaacgacaaagtcagccgtttcgattttatccgccagattgaagtggatggtcagcttatcaccttggagagcggtgaatttcaggtttataaacaaagccacagcgcgttgactgccctacagaccgaacaagagcaagatccagaacactccggcaagatggtggcaaaacgtcgtttccgcattggcgacatcgccggcgagcacaccgcgttcaaccagcttccggatggtaaagcagagtatcatggtaaggcgttttctagcgatgatgcaggcggcaaactgacgtacaccattgacttcgcgaaaaaacaaggtcatggtcgtatcgagcacctgaaaactccggagcagaatgttgaactggcggctgcggagctgaaggccgacgaaaagtcccacgctgttattctgggtgacacccgttatggtagcgaagaaaagggcacctaccacctggcgttgtttggtgaccgcgcacaggagatcgctggctctgcgaccgttaaaatcggagagaaggtgcatgaaatcggcattgcgggcaagcaataatga

SEQ ID NO: 35 - DNA, 1644 bp, synthetic construct
  source 1..1644: mol_type = other DNA
tcatctggtggggggggaagtggcggaggcggggtgaccgcagatatcggcaccggtctggctgacgcgctgactgcgcctctggatcacaaagacaagggcttgaagtccctgaccctggaagattcgatcagccagaacggcaccttgacgctgagcgcgcagggtgccgaaaaaacctacggaaacggtgacagcctaaacaccggtaaactgaagaatgataaagtgtctcgtttcgacttcattcgtcagattgaagtggacggccagctgatcaccttggagagcggcgagttccaagtttataaacaaagccatagcgcgttgacggcgctgcaaaccgaacaggagcaggatccggaacacagcgaaaaaatggttgctaagcgccgttttcgtattggcgacatagcaggcgagcacaccgcgtttaatcaactgccggacggcaaggccgagtatcatggcaaagccttcagcagcgacgacgctggtggtaaattgacgtacaccattgacttcgccgccaaacagggccacggcaagatcgagcacctgaagactccggaacagaacgtggagctggcagcagcggagctgaaggctgacgagaagagccacgccgtgattctgggcgatacccgttatggttctgaagaaaaaggtacataccatctggcgctgtttggtgatcgtgcacaagagatcgcgggttcggctaccgttaagatcggtgaaaaggtgcatgagatcgggatcgccggtaagcaaggcggctcgagcggttccggttctggcggcggcggcgttgcggcggacatcggtaccggcctggcggatgcgctgactgcgccactggatcataaagacaaaggtttgaagtccttgacgcttgaggacagcatttcacaaaacggtacgttaacccttagtgcgcaaggtgctgagaagacctttaaagttggtgacaaagataattccctgaacaccggtaagctcaagaacgataagatcagccgcttcgactttgttcagaaaatcgaggtggatggtcagaccattaccctggctagcggtgagttccagatttataaacaggaccactctgcggtcgtggccttacagatcgaaaagatcaacaacccggataagattgattcgctgattaaccaacgtagcttcctggttagcggtttaggtggtgagcacaccagcttcgacaaattgccgaaagacgtgatggcaacctaccgcggtactgcgttcggctctgatgatgcgggtggtaagttgacgtacacgatcgactttgcagcgaaacaaggtcatggcaaaatcgaacacctgaaatccccggaactgaatgttgatctggcagttgcatacatcaaaccggatgaaaagcaccacgcagtcatcagcggttccgtgctgtataatcaggatgagaaaggctcctatagcctgggtatttttggcgagaaggcgcaagaagtagctggtagcgcggaagttgaaaccgctaatggcattcatcacatcggcctcgctgcgaagcagggttctggtgggtcgggcgcacatattgttatggtggacgcgtacaagccgaccaaacatcaccaccaccatcattaatga

SEQ ID NO: 36 - DNA, 1626 bp, synthetic construct
  source 1..1626: mol_type = other DNA
tcatctgggggaggcggaagtggtggggggggcgttaccgcggacatcggtactggcctggccgacgccctgacggcaccgctggatcacaaagacaagggcttgaaatccttgactcttgaggattctatttcgcaaaacggcaccctgactttgagtgcgcagggtgcagagaagacctatggtaatggcgacagcttgaacaccggtaagctgaagaacgataaggtgagccgcttcgatttcatccgccagatagaagtagatggtcaactgattaccctggaaagcggtgaatttcaagtttataaacagagccattccgccttgaccgcgctgcaaaccgaacaagagcaagatccggaacattcggaaaagatggttgccaaacgtcgtttccgtattggcgacatcgcaggtgagcacaccgcgtttaatcagctgccggacggcaaagcggagtatcacggcaaggcgttcagcagcgacgacgcgggcggtaaactgacgtacaccattgatttcgctgcgaaacaaggtcatggtaagatcgaacacctgaaaacaccggaacaaaacgtggaattggcggctgcggagcttaaggcggacgagaagtcccatgcggtcatcctgggtgacacccgttacggctccgaagaaaaggggacgtaccacttggcgttgtttggtgatagagcacaggagatcgcgggcagcgcgaccgttaaaatcggcgagaaggttcatgaaattggtatcgccggtaagcagggttcgggtggtggcggggtggcagccgatatcggcaccgggcttgctgacgcgctcacggctccgctggaccacaaagacaagggtttaaagagcctgaccctggaagatagcatttcccagaacggcaccctgaccctgtctgcacaaggtgcggagaaaacctttaaagtaggtgataaggacaacagcctaaacaccggtaagctgaaaaatgacaagatctctcgtttcgactttgttcagaaaatcgaggtggatggtcagaccattaccttggctagcggcgagttccagatctataaacaagaccatagcgcggtcgtggcgttacagatcgagaagattaacaacccggataagatcgattcgctgattaaccagcgtagctttctggtttccggactcggtggcgagcacaccagcttcgacaagctgccaaaagacgtgatggcaacctaccgcggtacggctttcggttctgatgatgctggtggtaaactgacctacacgatcgacttcgccgcaaaacaaggccacggcaagattgagcacctgaaatccccggaactgaatgttgatctggcggttgcgtatattaaaccggatgaaaaacaccacgcagtcatttctggcagcgtgctgtacaatcaggatgagaagggtagctatagcctgggcatttttggtgagaaggcgcaggaggttgccggtagcgccgaagtggaaaccgctaatggtattcaccacatcggtctggccgctaaacagggcagcggtggctccggcgcacatatcgtgatggtggacgcatacaaaccgacgaaacatcatcatcaccaccactaatga

SEQ ID NO: 37 - DNA, 1611 bp, synthetic construct
  source 1..1611: mol_type = other DNA
gtggcagctgacatcggcactggtctggcggacgctctgaccgctccgctggaccacaaggacaaaggtttgaaaagcctgactttggaagattcgatctctcagaatggtacgctgaccctcagcgcgcaaggcgcggagaagacctttaaagttggtgataaggacaacagcttgaacaccggtaaactgaaaaacgataagattagccgcttcgacttcgtgcagaaaatcgaagtggacggtcagaccattacccttgcgagcggcgagttccagatttacaagcaggatcatagtgcggttgtcgcattacaaatcgaaaaaatcaataatccggataagattgattctctcatcaaccaacgtagcttcttggttagcggcctgggtggcgaacacaccagctttgataagctgccaaaagatgtcatggcaacctaccgtggtacggcgttcggctcggacgacgcgggtggcaaattaacttacaccattgactttgcagcgaagcagggccatggcaaaatcgagcacctgaagtccccggaactgaacgtggacctggcagtggcgtacatcaaaccggacgaaaagcatcatgctgtgatcagcggttcggtgctgtataaccaagatgagaaaggcagctatagcctgggtatttttggcgagaaggcgcaggaggtggcgggttccgccgaggttgaaaccgcgaatggcatccatcacattgggttggcggcaaaacagggctctagcggaggtggtggttccggtggtggcggtgttaccgcggacatcggtaccggtttggcggatgcgcttacggcaccgctggatcacaaagacaagggtctgaagtccttgaccttggaggactccatttcgcaaaacggcaccctgacgcttagcgctcaaggcgcagaaaagacctacggcaatggtgactcactgaacaccggtaaactgaagaacgacaaagttagccgcttcgactttatccgtcagattgaggttgatggtcagctgattaccctggaaagcggggagtttcaggtatataagcaatcccattccgcgctgactgccctgcagaccgaacaagaacaggacccggagcactccgaaaaaatggttgcaaagcgccgttttcgtattggtgacattgcgggcgagcacaccgcgttcaaccagctgcctgatggtaaagccgagtatcacggcaaggccttcagcagcgatgacgccgggggtaagttaacgtacaccattgactttgccgcgaagcaaggtcacgggaaaatcgagcacctgaagacaccggagcaaaatgtcgagttggctgcggcagagctgaaggctgacgaaaagagccatgcagtcatcctgggcgatacccgttatggttctgaagaaaagggtacgtaccacctggccttgttcggtgatcgtgcccaagagatcgcgggctctgctaccgttaaaatcggcgaaaaagtgcatgaaatcggtatcgcgggtaaacagggttctggcggctctggcgcccatattgttatggtggacgcatataaaccgaccaaacatcatcaccaccaccactaatga

SEQ ID NO: 38 - DNA, 1437 bp, synthetic construct
  source 1..1437: mol_type = other DNA
ttgaacaccggtaaactgaaaaacgataagattagccgcttcgacttcgtgcagaaaatcgaagtggacggtcagaccattacccttgcgagcggcgagttccagatttacaagcaggatcatagtgcggttgtcgcattacaaatcgaaaaaatcaataatccggataagattgattctctcatcaaccaacgtagcttcttggttagcggcctgggtggcgaacacaccagctttgataagctgccaaaagatgtcatggcaacctaccgtggtacggcgttcggctcggacgacgcgggtggcaaattaacttacaccattgactttgcagcgaagcagggccatggcaaaatcgagcacctgaagtccccggaactgaacgtggacctggcagtggcgtacatcaaaccggacgaaaagcatcatgctgtgatcagcggttcggtgctgtataaccaagatgagaaaggcagctatagcctgggtatttttggcgagaaggcgcaggaggtggcgggttccgccgaggttgaaaccgcgaatggcatccatcacattgggttggcggcaaaacagggctctagcggaggtggtggttccggtggtggcggtgttaccgcggacatcggtaccggtttggcggatgcgcttacggcaccgctggatcacaaagacaagggtctgaagtccttgaccttggaggactccatttcgcaaaacggcaccctgacgcttagcgctcaaggcgcagaaaagacctacggcaatggtgactcactgaacaccggtaaactgaagaacgacaaagttagccgcttcgactttatccgtcagattgaggttgatggtcagctgattaccctggaaagcggggagtttcaggtatataagcaatcccattccgcgctgactgccctgcagaccgaacaagaacaggacccggagcactccgaaaaaatggttgcaaagcgccgttttcgtattggtgacattgcgggcgagcacaccgcgttcaaccagctgcctgatggtaaagccgagtatcacggcaaggccttcagcagcgatgacgccgggggtaagttaacgtacaccattgactttgccgcgaagcaaggtcacgggaaaatcgagcacctgaagacaccggagcaaaatgtcgagttggctgcggcagagctgaaggctgacgaaaagagccatgcagtcatcctgggcgatacccgttatggttctgaagaaaagggtacgtaccacctggccttgttcggtgatcgtgcccaagagatcgcgggctctgctaccgttaaaatcggcgaaaaagtgcatgaaatcggtatcgcgggtaaacagggttctggcggctctggcgcccatattgttatggtggacgcatataaaccgaccaaacatcatcaccaccaccactaatga

SEQ ID NO: 39 - DNA, 1635 bp, synthetic construct
  source 1..1635: mol_type = other DNA
tctagcggaagtgggtcaggaggcggtggtgttgcggctgacatcggaaccggcctggcagacgcgttgaccgcgccgttggaccacaaagacaagggtttgaaaagcctgaccttggaagactcaatttcgcagaatggtaccctcacgctgagcgctcagggtgcggagaaaacgtttaaagttggtgacaaggacaacagcctgaacaccggtaaattgaagaacgataagattagccgttttgatttcgtgcagaaaatcgaggtggacggccaaaccattaccctggcgagcggcgagttccagatctacaagcaagaccattccgctgtcgtggccttacagattgaaaaaatcaacaacccggataagattgactccctgattaatcagcgtagcttcctggttagcggtctgggtggcgagcacaccagcttcgataagctgccaaaagatgttatggcaacctaccgcggtactgcgttcggttctgatgacgcgggcggtaagttgacctacaccatcgacttcgccgcgaaacaaggccacggcaagatcgagcacctgaaatctccggagctgaatgtggatctggcagtggcgtacattaaaccggacgagaagcaccacgcggttatttccggcagtgttctgtataaccaagatgaaaagggtagctatagcctgggcatctttggtgagaaggctcaagaagtggcgggctctgccgaagttgaaaccgctaatggcattcatcacattggtttggctgcgaaacaaggtggttcgggcggtgaggcagcggctaaagtcaccgctgacatcggcacgggcttggcggacgccctcacggctccgctggatcacaaggataagggcctgaagtccctaacgctggaagattccatttcacagaacggcacattgaccctgtccgcgcagggcgcagagaagacctacggcaatggagacagcctgaacaccggtaaactgaaaaacgataaagtgagccgcttcgacttcatccgtcagatcgaggtagacggtcagcttattacccttgaaagcggggagtttcaggtgtataaacaaagccattctgcactgactgcgctgcagaccgaacaggagcaggatccggaacactcggagaaaatggtggcaaaacgtcgtttccgcattggtgatatcgcgggcgaacacactgcgtttaatcaactgcctgacggcaaggcggaatatcatggtaaggccttcagcagcgatgacgcgggtggtaagttaacttacaccatcgattttgcagcgaaacaaggtcacggtaagatcgagcacctgaaaaccccggaacaaaacgtggaactggcagcggctgagctgaaggcggatgagaagagccatgcggttattctgggtgacacgcgttatggtagcgaagaaaagggtacgtaccatctggcgttatttggtgatcgtgcgcaagagatcgcaggctccgccaccgttaaaatcggtgaaaaggttcatgaaattgggatcgccggtaagcagggctctggcggctctggcgcacatatcgtgatggtcgacgcctataaaccgaccaaacatcaccatcaccatcactaatga

SEQ ID NO: 40 - DNA, 1635 bp, synthetic construct
  source 1..1635: mol_type = other DNA
tctagcgggtcaggaagtggcggaggtggagttgcggcagatataggcacgggcttggccgacgccctgacagctccactggaccacaaggataaagggctcaagtctttaacgcttgaggattccattagccaaaacggcaccctgactctgtccgctcagggtgcggaaaaaacttttaaagttggtgacaaagacaactctttgaacaccggcaaactcaaaaacgataagattagccgttttgacttcgtgcagaaaattgaagtcgacggccaaaccattaccctggcgtcaggcgagttccaaatttataaacaagaccactcggcggtggtggcgctgcaaattgagaagatcaacaacccggataaaattgatagcttgattaatcagcgttcgttcctggttagcggtctgggtggtgagcacacctcctttgataagttgccgaaagacgtgatggcaacctacagaggtaccgccttcggctcggatgatgcgggtggtaaattgacgtataccatcgatttcgccgcgaagcaaggtcatggtaagatcgagcacctgaagtccccggaactgaacgtggacctggctgttgcatacatcaaaccggacgagaaacaccacgcggtcatctccggttcagttctgtacaatcaggatgaaaagggtagctatagcctgggcatatttggtgaaaaagcgcaagaagtagcaggcagcgcggaggtggaaaccgctaatggcattcatcacatcggcttggctgcaaagcaggaggcggcagcgaaagaagcagctgcgaaggtgaccgcggacatcggcactggtctggctgatgccctcactgcgcctctggaccacaaggataagggtttgaagtccctcaccctggaggacagcatcagccaaaatggtacgctgaccctgagcgctcagggcgcggagaagacctacggtaatggtgattctctgaataccggtaagctgaagaacgacaaggtgtctcgcttcgacttcatccgtcagattgaggttgacggccagctgattaccttggaaagcggtgagttccaggtttataaacaaagccattccgcgctgaccgcgctgcaaaccgaacaggaacaggatccggagcacagcgaaaaaatggtcgcgaagcgccgctttcgtatcggtgatatcgcaggtgagcacaccgcctttaaccagctgccggatggcaaagcggagtatcatggtaaggcgtttagcagcgatgacgcgggaggtaagttgacctacacgatcgacttcgcagcgaagcagggtcacggtaagatcgagcacctgaagaccccggagcaaaacgttgaattggccgcggctgaactgaaagcggacgagaaatctcatgcagtgattctgggggacacccgttatggcagcgaggaaaaaggtacgtaccatctggcgttgtttggcgatcgtgcccaagaaatcgccggtagcgcgaccgttaaaatcggcgaaaaagttcatgagatcggcattgccggcaagcagggtagtggtggcagcggtgctcatatcgtgatggtagacgcttacaaaccgaccaaacaccatcatcaccaccactaatga

SEQ ID NO: 41 - DNA, 1602 bp, synthetic construct
  source 1..1602: mol_type = other DNA
agttcaggtggagggggagtagcagctgacatcggtgcaggcctcgcagacgcgctgaccgcgccgcttgatcataaggataagagcctgcagagcctgacattggatcagtccgtgcgtaaaaatgaaaagttgaagctagcggcccaaggtgcggaaaagacctacggcaacggcgactccttgaacaccggtaagctgaagaacgacaaggtgagcagattcgacttcatccgccagatcgaagtcgacggtcagctgattaccttggaatctggcgagtttcagatctataagcaggaccacagcgcggtcgtggccctgcagattgagaagatcaacaacccggataagatcgatagcttgatcaatcaacgtagcttcctggttagtggtttgggcggcgagcacacctcatttgacaaactgccaaaagatgttatggctacctaccgcggtacggctttcggctccgacgacgccggtggcaagctgacttacaccattgatttcgcagcaaaacaaggtcacggtaaaatcgagcacctgaaaagcccggagctgaacgtggatctggcggtagcttacatcaaaccggatgagaaacatcacgccgtcatcagcggttctgttctgtataaccaagatgagaaaggttcctatagcctgggcatttttggtgagaaagcgcaagaagttgcgggttctgcggaagtcgaaaccgccaatggtattcatcacatcggcctggcggcaaagcaaggcagcggcggtggcggggtgaccgctgatatcggcacgggtttagcggacgccctcacggctccgctggatcataaagacaaaggtctgaagtctttgaccctggaggattcaattagccagaacggtactctgacgctgagcgcgcagggggccgaaaagacctacggaaatggtgattctttgaataccggcaaactgaaaaacgataaagtttctcgcttcgactttatccgtcagattgaggtggacggccagctgattactctcgagtcgggcgagttccaggtttataaacaatcccattccgcgctgaccgcgctgcaaaccgaacaagagcaggatccggaacacagcgaaaagatggttgccaaacgtcgttttcgtattggtgacatcgcgggcgaacacaccgcgttcaaccagctgccgagcggtaaggctgagtatcacggcaaggcgtttagcagcgacgacgcaggtggtaagctgacgtacaccattgacttcgccgcgaaacaaggtcatggtaagattgagcatctgaaaactccggagcaaaatgttgaattggcgagcgctgagctgaaggcagatgaaaagagccacgcagtgattctgggtgacacccgttatggttcggaggaaaaaggcacctaccatctggcattgtttggcgaccgcgcacaggagatcgcgggttcggcgaccgttaaaattcgtgaaaaagttcatgaaatcggcatcgctggcaagcagggcagcggtggctccggagcgcatatcgtgatggtggacgcgtacaagccgaccaaacaccaccaccaccaccactaatga

SEQ ID NO: 42 - DNA, 1650 bp, synthetic construct
  source 1..1650: mol_type = other DNA
tctagcgggtcaggaagtggcggaggtggggtggcggccgacatcggcactggtttggcggacgcgctgacggctccgttggaccacaaagacaaaggtttgaagtccctgacgttagaggactcgatctctcagaacggtactctaacgctgagcgcgcaaggtgcagagaagacctttaaagtgggtgacaaggacaacagcttgaataccggtaaactgaagaacgacaagatcagcagattcgacttcgtccagaaaatcgaggtggacggccagaccattaccctggcgagcggtgagttccagatttataaacaagatcatagcgctgtcgtggcgctgcagattgagaagatcaacaacccggataagatcgacagcctgattaaccagcgtagctttctggttagcggtcttggcggcgaacacaccagctttgataaattaccgaaagatgtgatggcaacctaccgcggcactgcgtttggttctgatgatgcaggcggtaaactgacctacaccatcgacttcgcagccaagcaaggccacggtaagatcgagcacctgaagagcccggaattaaatgtcgacctggcggtggcatacattaaaccagacgaaaagcaccacgctgttatttctggtagtgttctgtataaccaggatgagaagggctcatattccctgggcatcttcggtgagaaggcgcaggaggtggccggttctgcggaggtggaaaccgcaaatggcattcatcacatcggtctggcggctaagcaagaagcagctgcgaaagaagcggcggcgaaagaagccgcggccaaggtcaccgcggacatcggcactggcctggctgatgctctgacagcaccgctggatcacaaagacaaaggcttgaagtcgctgaccttggaagatagcatctcgcaaaacggcaccctcacgttgagcgcgcagggtgcggaaaagacgtacggcaatggtgactccctcaacaccggcaaattgaagaatgataaggtgagccgttttgacttcatccgtcagattgaagttgacggtcagctgattaccctggagagcggtgaatttcaggtttataaacaaagccattctgcgttaacggctctgcaaaccgaacaagagcaggatccggaacacagcgaaaagatggttgcgaagcgccgttttcgtattggcgatatcgccggtgagcacaccgcgtttaatcaactgccggacggcaaagcggaatatcatgggaaagcattcagcagcgatgatgcgggtggcaagttgacctacaccatcgatttcgccgcgaagcagggtcatggtaagattgagcacctgaaaaccccggaacaaaacgttgagctggcggcggcggagttaaaagcggacgagaaaagccacgccgtgattctgggtgatacccgttatggctccgaggaaaagggtacgtaccatctggccctcttcggcgatcgcgctcaggagattgctggttcggcgaccgttaaaatcggtgagaaagttcatgaaatcggcattgcaggtaaacaaggctccggcggttccggcgcacatattgttatggtagatgcgtacaagccgaccaaacatcaccaccatcaccattaatga

SEQ ID NO: 43 - DNA, 1665 bp, synthetic construct
  source 1..1665: mol_type = other DNA
tctagcgggtcaggaagtggcggaggtggggtggcggcggacatcggcaccggtcttgcggatgcgctgaccgctccactggatcataaagacaaaggtctgaagtctctgaccttggaggattctattagccagaacggtacgttgactctgagcgcgcagggtgctgaaaagacttttaaagtgggtgacaaggataatagcttgaacaccggtaagctcaagaacgacaagatctcccgcttcgactttgttcagaaaatcgaggtggacggccagacgattaccctggcgagcggtgagttccagatttataaacaagatcattccgcggttgttgcactgcagatcgagaagattaacaacccggataagatcgattctctgatcaatcagcgtagctttctggttagcggtctcggtggtgagcacacttcatttgacaagctgccgaaagacgtgatggccacgtaccgcggtacagccttcggcagcgacgacgctggcggtaaactgacgtacaccattgacttcgccgctaaacagggtcacggtaaaatcgagcacctgaaaagcccggaactgaatgttgatctggcagtggcgtatattaaaccggacgagaaacaccacgcggtcatctcgggctctgttctgtacaatcaggacgaaaagggttcctatagcttgggtatttttggtgagaaagcccaagaagtggcgggctctgctgaggtcgaaaccgcgaatggcattcatcacatcggcctggctgcgaagcaagaggctgcagccaaagaagccgccgcgaaagaggcggctgcgaaagaagccgcggcgaaggtcaccgcggatatcggcacgggtctggctgacgcgcttaccgctccgctggaccacaaggacaaaggtttgaagtccttaaccctggaagattccatcagccaaaacggtaccttgaccttaagcgcgcaaggtgcggaaaagacctacggaaacggcgacagcctgaataccggcaagttgaaaaacgataaggtgagcagattcgacttcattcgtcagattgaggttgatggtcagctgattaccctggagagcggcgagtttcaagtctataaacaatcccatagcgcattgactgcgctacaaaccgaacaagaacaggatccggagcacagcgaaaaaatggttgcgaaacgtcgtttccgcattggcgacatcgccggtgagcacaccgcattcaaccagctgccggatggcaaggccgaatatcatggtaaggcgtttagcagcgatgatgcaggcggtaaattgacgtacaccatcgacttcgctgcaaagcagggtcacggcaagatcgagcacctgaagacccctgaacaaaacgtggagctggcggcagccgaactgaaggctgatgaaaaaagtcatgcagttatcctgggcgacacccgttatggttcggaggaaaagggcacgtaccacctggcgttgtttggcgatcgtgcacaggagattgcaggttctgcgaccgtaaaaatcggtgaaaaggtgcatgaaattggtatcgcaggtaagcaaggctcaggaggctctggcgcgcatatcgtgatggttgatgcatacaaaccgaccaaacatcatcaccaccaccactaatga

SEQ ID NO: 44 - DNA, 1614 bp, synthetic construct
  source 1..1614: mol_type = other DNA
agttcaggtggagggggagtagcagctgacatcggtgctggcttggcggatgccctgaccgcgcctctggatcacaaagacaaaagcctgcagtcgctgaccctggaccagagcgttcgtaaaaatgaaaagttgaagttggctgcccagggcgccgagaaaacctacggcaacggcgattcgcttaacaccggtaagttgaagaacgacaaagtctcacgtttcgatttcatccgtcagattgaagtggacggtcaactgatcaccctggaatctggcgagttccagatctataaacaggaccactctgctgtggttgcactgcaaatcgagaagatcaacaacccggataaaatcgacagcctgattaaccagcgtagcttcttggtttctggtctgggtggtgagcacacttcgtttgataaactgccgaaggatgttatggctacctaccgcggtacagcgttcggctccgacgacgcgggcggtaaactcacgtacaccattgactttgcggctaagcaaggtcatggtaagattgagcacctgaagagcccggagctgaacgtggacctggcggtggcatacattaaaccggatgagaagcaccatgcggtgatcagcggttccgtgctgtataaccaggacgagaaaggctcctacagcctcggtatttttggcgaaaaggcgcaggaggtggccggtagcgctgaggttgaaaccgcgaatggaatccatcacatcggcctggcggcaaaacaggaggctgctgcaaaagaagcagcggcgaaggtcaccgcagacattggtacgggtttagctgatgccctgactgcgccactggatcacaaagataagggtcttaagtccctgacgttagaagattccatcagccagaacggtacgctgacgctgagcgcgcaaggcgcagagaaaacctacggtaatggcgactctttaaataccggtaagctgaagaatgataaagtttctcgcttcgacttcatacgccagattgaggtcgacggccaactgattaccctggagagcggagaatttcaagtgtataaacaaagccatagcgctttgaccgcgctccaaaccgaacaagagcaagatccggaacactccgaaaaaatggtggcgaaacgtcgttttcgtattggcgacattgcgggtgagcacacggccttcaaccagcttccgagcggcaaggcggaatatcatggtaaagcgtttagcagcgatgatgcgggtggtaaattgacttacaccatcgacttcgcagcgaagcaaggtcatggtaagatcgagcacctgaagaccccggaacagaatgttgaattggcgagcgcggagctgaaagcagacgagaagtcccatgctgtgatcctgggcgacacccgttatggcagcgaggaaaagggcacctaccatctggcgttgtttggtgatagagcccaagagatcgcaggctctgctaccgtaaaaatccgcgaaaaggttcatgaaattgggatcgctggcaagcagggtagcggtggcagtggcgcgcatattgttatggttgacgcgtataagccgaccaaacaccaccaccatcaccactaatga

SEQ ID NO: 45 - DNA, 1629 bp, synthetic construct
  source 1..1629: mol_type = other DNA
tcaagtggtggaggaggggtagcagctgacatcggtgcgggattggcagatgcgcttacggcgccactggaccacaaagataaaagcctccaatcgctgaccttagaccagtccgttcgtaaaaacgaaaagctcaagctggccgcccaaggtgcagagaagacgtacggaaacggcgactcattgaataccggtaagctgaagaacgataaagtgtcccgcttcgacttcatccgtcagattgaagtggacggccagctgatcaccttggagtcaggcgagttccagatttacaagcaagatcatagcgcggtcgtggctcttcaaattgagaaaatcaacaacccggacaagatcgactccctgatcaatcagcgtagctttctggtttccggtctgggcggtgaacataccagcttcgataaattgccgaaagacgttatggctacctaccgcggtacggccttcggttccgacgatgcgggtggtaaactgacctacaccattgatttcgcagcaaaacagggccacggcaagattgagcacctgaagagtccggaactgaacgtcgacctggcggtggcgtacattaaaccggatgaaaagcaccacgccgtcattagcggttccgtgctgtataaccaagacgagaaaggttcttatagcctaggtatctttggtgagaaggctcaagaggttgctggttctgctgaggtggaaaccgctaatggtatccatcacattggcctagcggctaagcaggaggccgcagccaaagaggctgccgcgaaagaagcagctgcgaaagtcaccgctgatatcggtactggtctggcagatgcgttgaccgcaccgctggatcacaaggacaagggtcttaagtcgctgactctggaagattcgattagccagaatggcaccctgacgctgagcgcgcaaggtgcagaaaaaacctacggcaacggcgactctttgaataccggtaagctgaagaacgacaaagtttccagattcgactttatccgccagatcgaggttgatggtcaactgattaccctggagagcggtgagttccaggtttataagcagagccacagcgcgttgacggcgctccaaaccgaacaggagcaggatccggaacactctgaaaagatggtggctaaacgtcgttttcgtatcggcgacatcgcgggcgaacacaccgcttttaatcagctgccgagcgggaaagcggagtatcatggcaaagcgtttagcagcgatgatgcgggtggtaaactgacgtacaccattgacttcgcggccaaacagggtcatggcaagatcgagcatctgaagactccggaacaaaacgtggaactggcgagcgcggaactgaaagcggacgagaaaagccatgcggtgatcttgggtgatacccgttatggcagcgaggaaaagggtacgtaccatctggctttgtttggtgatcgtgcacaggagatcgccggttctgcgaccgttaaaatccgcgaaaaggtgcatgaaataggcattgcaggcaagcaaggctctggcggcagcggcgcgcatattgttatggttgacgcatataaaccgaccaaacaccaccaccaccaccattaatga

SEQ ID NO: 46 - DNA, 1644 bp, synthetic construct
  source 1..1644: mol_type = other DNA
agttcaggtggagggggagtagcagctgacatcggcgctggccttgctgatgcgctcacggctccgctggatcacaaagacaagtccctgcaatccttgacgctcgaccagagcgttcgtaaaaacgaaaagttgaagctggcggcacagggcgcggagaagacttacggcaacggtgactccttgaacaccggcaagctgaagaatgataaagtatcccgttttgactttatacgtcaaatcgaggtggacggtcagctgattacccttgagagcggcgagttccaaatctacaaacaagaccatagcgcagttgttgccctgcagattgagaagatcaacaacccggataagatcgatagcctgatcaatcaacgtagcttcctggtgtctggtctgggtggtgaacacaccagctttgacaaacttccgaaagatgttatggcaacctaccgcggtactgccttcggctctgatgatgcgggcggtaaattaacctataccattgactttgctgcgaaacaaggtcatggtaagatcgagcacctgaagtctccggaattgaacgttgatctggcggtcgcgtacatcaaaccggatgaaaaacaccacgcagtcatctctgggtccgtgctgtataaccaggatgagaaaggctcttatagcctgggtatttttggtgagaaggcccaagaggttgcgggttccgcggaggtggaaaccgctaatggtattcatcacattggcttggcagccaaacaagaagcagcggcgaaagaagcggcggcgaaagaggccgcggccaaagaagcagcggctaaagtcaccgcggacattggcaccggtctggcggatgcgctgactgcaccactggaccataaagacaagggtttgaagagcttgacgctggaagatagcatcagccagaacggcaccttgaccttatcagcgcagggcgcggagaaaacctacggtaatggcgacagcctgaacactggcaagctgaagaacgataaggtgagccgtttcgacttcatccgccaaattgaggtggacggccagctgattaccctggaaagcggtgagttccaggtgtataagcagagccatagtgcattaacggcgctgcagaccgaacaagaacaggatccggagcactcggaaaagatggttgccaaacgtcgtttcagaattggcgatatcgccggcgagcataccgcctttaatcagctgccaagcggtaaggcggagtatcacggcaaagcgttcagcagcgacgacgcaggcggcaaattgacctacaccattgacttcgccgctaaacagggtcatggtaaaatcgagcacttgaagaccccggagcagaatgttgaactggctagcgctgagctgaaggccgacgaaaagagccatgcagtgattctgggtgatacccgttatggttctgaagaaaagggtacgtaccatctggcgctgtttggtgaccgcgcacaggagatcgctggttcggcgaccgttaaaattcgcgaaaaggtgcacgaaatcggcatcgcaggcaagcaaggttccggtggctccggcgcgcatatcgtgatggttgacgcgtacaaaccgacgaaacaccaccaccaccaccactaatga

SEQ ID NO: 47 - protein, 13 aa, synthetic construct
AHIVMVDAYKPTK

SEQ ID NO: 48 - protein, 92 aa, synthetic construct
DSATHIKFSKRDEDGKELAGATMELRDSSGKTISTWISDGQVKDFYLYPGKYTFVETAAPDGYEVATAITFTVNEQGQVTVNGKATKGDAHI

SEQ ID NO: 49 - protein, 9 aa, synthetic construct
GGSGGSGGS

SEQ ID NO: 50 - protein, 12 aa, synthetic construct
GGSGGSGGSGGS

SEQ ID NO: 51 - protein, 205 aa, synthetic construct
MKMEELFKKHKIVAVLRANSVEEAKKKALAVFLGGVHLIEITFTVPDADTVIKELSFLKEMGAIIGAGTVTSVEQARKAVESGAEFIVSPHLDEEISQFAKEKGVFYMPGVMTPTELVKAMKLGHTILKLFPGEVVGPQFVKAMKGPFPNVKFVPTGGVNLDNVCEWFKAGVLAVGVGSALVKGTPVEVAEKAKAFVEKIRGCTE

SEQ ID NO: 52 - protein, 310 aa, synthetic construct
MDSATHIKFSKRDEDGKELAGATMELRDSSGKTISTWISDGQVKDFYLYPGKYTFVETAAPDGYEVATAITFTVNEQGQVTVNGKATKGDAHIGGSGGSGGSGGSMKMEELFKKHKIVAVLRANSVEEAKKKALAVFLGGVHLIEITFTVPDADTVIKELSFLKEMGAIIGAGTVTSVEQARKAVESGAEFIVSPHLDEEISQFAKEKGVFYMPGVMTPTELVKAMKLGHTILKLFPGEVVGPQFVKAMKGPFPNVKFVPTGGVNLDNVCEWFKAGVLAVGVGSALVKGTPVEVAEKAKAFVEKIRGCTE

SEQ ID NO: 53 - protein, 6 aa, synthetic construct
GSGGSG

SEQ ID NO: 54 - protein, 139 aa, synthetic construct
SSGGGGSGGGGVTADIGTGLADALTAPLDHKDKGLKSLTLEDSISQNGTLTLSAQGAEKTYGNGDSLNTGKLKNDKVSRFDFIRQIEVDGQLITLESGEFQVYKQSHSALTALQTEQEQDPEHSEKMVAKRRFRIGDIA

SEQ ID NO: 55 - protein, 134 aa, synthetic construct
GSGGGGVTADIGTGLADALTAPLDHKDKGLKSLTLEDSISQNGTLTLSAQGAEKTYGNGDSLNTGKLKNDKVSRFDFIRQIEVDGQLITLESGEFQVYKQSHSALTALQTEQEQDPEHSEKMVAKRRFRIGDIA

SEQ ID NO: 56 - protein, 128 aa, synthetic construct
VTADIGTGLADALTAPLDHKDKGLKSLTLEDSISQNGTLTLSAQGAEKTYGNGDSLNTGKLKNDKVSRFDFIRQIEVDGQLITLESGEFQVYKQSHSALTALQTEQEQDPEHSEKMVAKRRFRIGDIA

SEQ ID NO: 57 - protein, 120 aa, synthetic construct
GEHTSFDKLPKDVMATYRGTAFGSDDAGGKLTYTIDFAAKQGHGKIEHLKSPELNVDLAVAYIKPDEKHHAVISGSVLYNQDEKGSYSLGIFGEKAQEVAGSAEVETANGIHHIGLAAKQ

SEQ ID NO: 58 - protein, 134 aa, synthetic construct
SSGGGGVAADIGAGLADALTAPLDHKDKSLQSLTLDQSVRKNEKLKLAAQGAEKTYGNGDSLNTGKLKNDKVSRFDFIRQIEVDGQLITLESGEFQIYKQDHSAVVALQIEKINNPDKIDSLINQRSFLVSGLG

SEQ ID NO: 59 - protein, 119 aa, synthetic construct
GEHTAFNQLPDGKAEYHGKAFSSDDAGGKLTYTIDFAAKQGHGKIEHLKTPEQNVELAAAELKADEKSHAVILGDTRYGSEEKGTYHLALFGDRAQEIAGSATVKIGEKVHEIGIAGKQ

SEQ ID NO: 60 - protein, 141 aa, synthetic construct
SSGSGSGGGGVAADIGTGLADALTAPLDHKDKGLKSLTLEDSISQNGTLTLSAQGAEKTFKVGDKDNSLNTGKLKNDKISRFDFVQKIEVDGQTITLASGEFQIYKQDHSAVVALQIEKINNPDKIDSLINQRSFLVSGLG

SEQ ID NO: 61 - protein, 137 aa, synthetic construct
GSGGGGVAADIGTGLADALTAPLDHKDKGLKSLTLEDSISQNGTLTLSAQGAEKTFKVGDKDNSLNTGKLKNDKISRFDFVQKIEVDGQTITLASGEFQIYKQDHSAVVALQIEKINNPDKIDSLINQRSFLVSGLG

SEQ ID NO: 62 - protein, 131 aa, synthetic construct
VAADIGTGLADALTAPLDHKDKGLKSLTLEDSISQNGTLTLSAQGAEKTFKVGDKDNSLNTGKLKNDKISRFDFVQKIEVDGQTITLASGEFQIYKQDHSAVVALQIEKINNPDKIDSLINQRSFLVSGLG

SEQ ID NO: 63 - protein, 73 aa, synthetic construct
LNTGKLKNDKISRFDFVQKIEVDGQTITLASGEFQIYKQDHSAVVALQIEKINNPDKIDSLINQRSFLVSGLG

SEQ ID NO: 64 - protein, 119 aa, synthetic construct
GEHTAFNQLPSGKAEYHGKAFSSDDAGGKLTYTIDFAAKQGHGKIEHLKTPEQNVELASAELKADEKSHAVILGDTRYGSEEKGTYHLALFGDRAQEIAGSATVKIREKVHEIGIAGKQ

SEQ ID NO: 65 - DNA, 417 bp, synthetic construct
  source 1..417: mol_type = other DNA
tctagcggaggtggtggttccggtggtggcggtgttaccgcggacatcggtaccggtttggcggatgcgcttacggcaccgctggatcacaaagacaagggtctgaagtccttgaccttggaggactccatttcgcaaaacggcaccctgacgcttagcgctcaaggcgcagaaaagacctacggcaatggtgactcactgaacaccggtaaactgaagaacgacaaagttagccgcttcgactttatccgtcagattgaggttgatggtcagctgattaccctggaaagcggggagtttcaggtatataagcaatcccattccgcgctgactgccctgcagaccgaacaagaacaggacccggagcactccgaaaaaatggttgcaaagcgccgttttcgtattggtgacattgcg

SEQ ID NO: 66 - DNA, 402 bp, synthetic construct
  source 1..402: mol_type = other DNA
ggcagcggaggtggcggtgttaccgcggacattggtactggtttggcggacgctctgactgcgccactggaccacaaagataagggcttgaagtcattgaccttggaggatagcattagccaaaatggcaccctgacactgtctgcgcagggtgccgagaagacctacggtaatggggactctctgaacactggcaaacttaaaaacgataaggtgagccgcttcgattttatccgtcaaattgaagtggacggtcagctgattacgctggagagcggcgagtttcaggtttataaacaaagccattccgctctgacggctttgcaaaccgaacaagaacaggacccggagcactctgaaaagatggtggctaaacgtcgtttccgtattggcgacattgca

SEQ ID NO: 67 - DNA, 384 bp, synthetic construct
  source 1..384: mol_type = other DNA
gtgaccgcggacatcggcactggtctggctgatgccctcactgcgcctctggaccacaaggataagggtttgaagtccctcaccctggaggacagcatcagccaaaatggtacgctgaccctgagcgctcagggcgcggagaagacctacggtaatggtgattctctgaataccggtaagctgaagaacgacaaggtgtctcgcttcgacttcatccgtcagattgaggttgacggccagctgattaccttggaaagcggtgagttccaggtttataaacaaagccattccgcgctgaccgcgctgcaaaccgaacaggaacaggatccggagcacagcgaaaaaatggtcgcgaagcgccgctttcgtatcggtgatatcgca

SEQ ID NO: 68 - DNA, 360 bp, synthetic construct
  source 1..360: mol_type = other DNA
ggcgaacacaccagctttgataagctgccaaaagatgtcatggcaacctaccgtggtacggcgttcggctcggacgacgcgggtggcaaattaacttacaccattgactttgcagcgaagcagggccatggcaaaatcgagcacctgaagtccccggaactgaacgtggacctggcagtggcgtacatcaaaccggacgaaaagcatcatgctgtgatcagcggttcggtgctgtataaccaagatgagaaaggcagctatagcctgggtatttttggcgagaaggcgcaggaggtggcgggttccgccgaggttgaaaccgcgaatggcatccatcacattgggttggcggcaaaacag

SEQ ID NO: 69 - DNA, 402 bp, synthetic construct
  source 1..402: mol_type = other DNA
agttcaggtggagggggagtagcagctgacatcggtgcaggcctcgcagacgcgctgaccgcgccgcttgatcataaggataagagcctgcagagcctgacattggatcagtccgtgcgtaaaaatgaaaagttgaagctagcggcccaaggtgcggaaaagacctacggcaacggcgactccttgaacaccggtaagctgaagaacgacaaggtgagcagattcgacttcatccgccagatcgaagtcgacggtcagctgattaccttggaatctggcgagtttcagatctataagcaggaccacagcgcggtcgtggccctgcagattgagaagatcaacaacccggataagatcgatagcttgatcaatcaacgtagcttcctggttagtggtttgggc

SEQ ID NO: 70 - DNA, 357 bp, synthetic construct
  source 1..357: mol_type = other DNA
ggcgagcacaccgcgttcaaccagctgcctgatggtaaagccgagtatcacggcaaggccttcagcagcgatgacgccgggggtaagttaacgtacaccattgactttgccgcgaagcaaggtcacgggaaaatcgagcacctgaagacaccggagcaaaatgtcgagttggctgcggcagagctgaaggctgacgaaaagagccatgcagtcatcctgggcgatacccgttatggttctgaagaaaagggtacgtaccacctggccttgttcggtgatcgtgcccaagagatcgcgggctctgctaccgttaaaatcggcgaaaaagtgcatgaaatcggtatcgcgggtaaacag

SEQ ID NO: 71 - DNA, 423 bp, synthetic construct
  source 1..423: mol_type = other DNA
tctagcggttcaggaagtggcggagggggggtggcagctgacatcggcactggtctggcggacgctctgaccgctccgctggaccacaaggacaaaggtttgaaaagcctgactttggaagattcgatctctcagaatggtacgctgaccctcagcgcgcaaggcgcggagaagacctttaaagttggtgataaggacaacagcttgaacaccggtaaactgaaaaacgataagattagccgcttcgacttcgtgcagaaaatcgaagtggacggtcagaccattacccttgcgagcggcgagttccagatttacaagcaggatcatagtgcggttgtcgcattacaaatcgaaaaaatcaataatccggataagattgattctctcatcaaccaacgtagcttcttggttagcggcctgggt

SEQ ID NO: 72 - DNA, 411 bp, synthetic construct
  source 1..411: mol_type = other DNA
ggttcgggtggtggcggggtggcagccgatatcggcaccgggcttgctgacgcgctcacggctccgctggaccacaaagacaagggtttaaagagcctgaccctggaagatagcatttcccagaacggcaccctgaccctgtctgcacaaggtgcggagaaaacctttaaagtaggtgataaggacaacagcctaaacaccggtaagctgaaaaatgacaagatctctcgtttcgactttgttcagaaaatcgaggtggatggtcagaccattaccttggctagcggcgagttccagatctataaacaagaccatagcgcggtcgtggcgttacagatcgagaagattaacaacccggataagatcgattcgctgattaaccagcgtagctttctggtttccggactcggt

SEQ ID NO: 73 - DNA, 393 bp, synthetic construct
  source 1..393: mol_type = other DNA
gtggcagctgacatcggcactggtctggcggacgctctgaccgctccgctggaccacaaggacaaaggtttgaaaagcctgactttggaagattcgatctctcagaatggtacgctgaccctcagcgcgcaaggcgcggagaagacctttaaagttggtgataaggacaacagcttgaacaccggtaaactgaaaaacgataagattagccgcttcgacttcgtgcagaaaatcgaagtggacggtcagaccattacccttgcgagcggcgagttccagatttacaagcaggatcatagtgcggttgtcgcattacaaatcgaaaaaatcaataatccggataagattgattctctcatcaaccaacgtagcttcttggttagcggcctgggt

SEQ ID NO: 74 - DNA, 219 bp, synthetic construct
  source 1..219: mol_type = other DNA
ttgaacaccggtaaactgaaaaacgataagattagccgcttcgacttcgtgcagaaaatcgaagtggacggtcagaccattacccttgcgagcggcgagttccagatttacaagcaggatcatagtgcggttgtcgcattacaaatcgaaaaaatcaataatccggataagattgattctctcatcaaccaacgtagcttcttggttagcggcctgggt

SEQ ID NO: 75 - DNA, 357 bp, synthetic construct
  source 1..357: mol_type = other DNA
ggcgaacacaccgcgttcaaccagctgccgagcggtaaggctgagtatcacggcaaggcgtttagcagcgacgacgcaggtggtaagctgacgtacaccattgacttcgccgcgaaacaaggtcatggtaagattgagcatctgaaaactccggagcaaaatgttgaattggcgagcgctgagctgaaggcagatgaaaagagccacgcagtgattctgggtgacacccgttatggttcggaggaaaaaggcacctaccatctggcattgtttggcgaccgcgcacaggagatcgcgggttcggcgaccgttaaaattcgtgaaaaagttcatgaaatcggcatcgctggcaagcag